European Patent Application EP 4 748 935 A1, published May 27, 2026. Title: Composition for providing bacteria with environmental stress resistance. Applicant: KABUSHIKI KAISHA YAKULT HONSHA. The sequence listing filed with the application follows.

SEQUENCE LISTING (32 sequences)

SEQ ID NO: 1 - DNA, 930 bp, Lacticaseibacillus paracasei
  source 1..930: mol_type = other DNA
atgaacgagcaaatcgacctttcacggctgtggaatgtgtttaaacgcagctttattgcaatggttatccttggcattttatgtatggttgcggcttattttggtgcgaagacttttattgtaccaaaatacgaagctgacacttcgctgttggtcaaccgcaagcaggataatgatccaaatatgcagttgaatgcacaacaagctgatgtgcagatcattaatacttataaagatattattacgcgtccggttgtattacaggctgttgctggtgatttgacaagtccgcggcgcgtgataaccaagaaagctgaaaaagcagtttatggtacgcgatataatgcgacgaccggcattcgtgaacggtatgttgtggaaaaagccaaaccagctcagtacaaactaaaaccagcaaaatattcaaacttaacagcggatgatctagccaaaatggtttcggtatcaacccaacaaaattctcaagtgtttacggttagtgtcaaggatactgatccaattcgagcgcgtgatatagcaaatgaagttgccaaggtatttaaacaaaaaattgcccaaatcatgagtatttccaacgtctctattgtttcggaggcttcggctaacctatcgccggtttcaccgaagttaccattgattgcccttgtagggttacttttaggcatactggttgcattcatctggggattaattcgagagcttacagaccaaaccattaaagaccttgactttattactgatgatttgggtttagtcaatcttggcatcgtaaattatgttaagcgcatgaaagacatggaccaagcgattgcgaaggttaaatctgaaaatgaagagtcaaaagacgatgaatcttttgaagaattcaatatgcaggatttacctcagcgcagccgtcgccggatttga

SEQ ID NO: 2 - DNA, 759 bp, Lacticaseibacillus paracasei
  source 1..759: mol_type = other DNA
atgagcttgaatgggatttttaaaaaattcacgcatcgtgatgaagaagataatgaaacacagaaaaacggtgttatgttggttacttttgcagagccaaaacatgttgttgctgaacagtttcgaacagtgagaacgaatattgagtttgctggggctgcattagatcgatgtgaagtcgtaatgttcacttcttcaagcatgtctgaagggaagtcaactgtttcggcaaacgttgctgtaacttgggctcaagcgggggaaaaagttttattgattgatgcagatttacgtagaccgacagttcatgctacttttagaacgctcaaccttgaaggggttacgactgtattaacggggaaaactaaaccatcagatgttgtagaaaaaacatttgtcgacaatctcgacattattacatccggcccagtgccaccaaatccctcagaacttttaaattcaaagcgtatggcaaatttgttggaatggggtcgagcaaattatgacatcattgttttagatgctccttcagttttggcagtatcagatgtacaggtgttagttccaaagactgacggggttgttgtcgtaacaaacatgggaaaaaccttaaaaggtgatttgaagagaactgttgaggtcttgaagctggcaaaggcaaaaattcttgggtctgtcgaacgagtgcgcgctacgaagggcgatcgcggttatggctatggttatggttacgggtatcaaagtaacgatgagcgttag

SEQ ID NO: 3 - DNA, 1182 bp, Lacticaseibacillus paracasei
  source 1..1182: mol_type = other DNA
gtgacagagaagcgtaaggtatttatcattggatcaaaaggtacaccagcaaaatatggtggctttgagacgttcgtagacaatttagtttctcgtcagaatagcagtcaaattaaatactttattgcctgtcgaagagacttatccgacaataaagcggatttatatgactataaaaaagcaacttgttttaatgttgatgttcccaatataggacctgccaaagcaattttgtatgatcttcgtgctttgtcttggacgttagactatattcagaagaataacattaggggagcaattgtttatattcttgcttgtcgggttggtcctttcttaaagcattatagtaaacggcttaaactttacgacacacaaatttttgtgaatccggatggtcacgaatggatgagggccaagtggggattttttgttaggaaatactggaagttatctgaacggttaatgattaaagatgcagatttgatcatctgtgatagtaaacacattgaactgtatattcgggaaaaatatcgcagttacaaaccaaagacgatatattcatcatatggcgccgatgttgccacctcacaagacgtgaaagcacaagatcttcaaaactggtttaataaaaagcagattagttcaggtcagtactatctagttgtgggtagatttgtaccagaaaataattaccaaacaattgttgctgaatttgaaaaatccaaaaccaaaaaggatttggtaatcataacaaatcccgataataccaagttcttgaaatcacttaaagaccaaactggctttgaaaaagataacagaattaaatttgttggcactgtgtatgacaaggaccttttatctgcaatcaggagaaatgcatttggatacatccatgggcatgaagtgggcggaactaatccctctttattggaagctttgggaaccacaaatctaaacttgctgttcgatgttgggttcaacaaagaagtggggcaggatgctgctgtttactggaataagcaggctggcaatttagcccatattattaatagagtggatcaaatgtcggaagaagaacgtcaaacccttggcaaaaaggccaagcagatcattgacaaaaacttctcctgggataagatagtaagtcaaaatgaaagacaatttatcgatggaaaaatataa

SEQ ID NO: 4 - DNA, 1158 bp, Lacticaseibacillus paracasei
  source 1..1158: mol_type = other DNA
atggaaaaatataagattctctttcttcatgcaggtgcagaattatatggtgcagataagattttattggagatagtagagaatatagaccgtaaaactttcgagccaatcgttattttgccggaagacggtccattggtttcaaagatgagagaagcaggggccgaagttagcgtcttgccatatccgattcttcggcgaaagtttttcaacatacgaggtatcggtaactacatctttagctatattaggttctccagacgcttgaaaaaaattgtcaataaagagaacattagacttgttcacgtcaatacgacagccgttttagaaggtgtttggctaaaactttttacaaaggctaaaattgtttggcatgttcacgaaatcatcatgaagcccaaatttatttacaaactgatttgttttctcatacagcacttttctgatcaggcagttgctgtatcagatgcaacaaaacaaagactcattgattccggaatcgttgataagatgaaagtaattaccattcataatggtataagtaaagattacccgcaaaatgggccggattatgtgcgaaaatctttgagcatctctccagatgcagttgtcattggaatggttggaagagtgaacgcttggaagggccaaggggatttcatagatgctgtaggtcccattttacaaaaaagtcaaaatgttcatgctctcctcgtggggagtgcttatcagggagaagaagtttatgagcacaagctgttcgacaaagtagcttctttggataccaaggaacgtatacacctctgtccctttaccgaacagattgctgattactattcggctttcaacattttcgtactccctagcatccagcctgatccttttccaacagttgtcttagaggcaatgtcaaattcgttgcctgttgtcgcatatgatcacgggggagctagtgagatgattgtggacaatgagaccggttatctctgcactgctttggacgtctctgaattaagtcggaaactagagttactggttggagatcgtgcacttcggataaaaatgggacaaaaagccagagttcgacaagaagctgagttcagtttagatcaattcgtgaacagaatgacaagggtatacctcgacctgattgaatga

SEQ ID NO: 5 - DNA, 975 bp, Lacticaseibacillus paracasei
  source 1..975: mol_type = other DNA
gtgacagtgaatcgaaaaacagacgtctctattattattcccgcccataatgcagagcctttcattacaaagtgtctccaaagcatccaacagcaaagttttcacaactttgaagttctagttgtagagaatggttcaacggatcataccgtcgaaagtgttttaccttttgtttcgacagacaaaaggatcagattattgcaaaattcagatcttggagtcagtaacgcaagaaacttagctttacagaaagctcaatctaaatttgttacatttgttgatgctgatgactacatatcgaatactcacattcaggttttgatggatagtgtaaaagataaagaagacgacatgggtgttactggattttcttatgaaaccgaggacgggaaaattttaaaagtaatttccgttttaaattcaaagatgagtgcagaagaggcaataagagctacctatgaccttactggaattcaaggaattgtcagcaacaagatctttaagaagtcaataatagatcgatacggtatacgatttgatccctccatctctaaatatgaagaccataagtttgttgtggcgtatttagtccattgtcaacaggtttcttgtaagagtgacataacttaccattatatcaaacatccagagagttctttgttcacggtaaagaccagtttgattcaagatttagatgtctttttgtcgattcgaaaaatgattgttaatcatggatttaaggactttaaaaagtatgtaaatgatccgctacaaaacatagttctaagtcattattggcatccagttgattctcatgataaaaccgaagctgctaaaaggatggttgatagaaagtttttctcatacaatctgctcaatatgtcaatcaaaaataaattgaaatgcttttttgcttttctttctttaggtccgtattgtattaagcggaaatttcgcaataatgatgcatcatga

SEQ ID NO: 6 - DNA, 1260 bp, Lacticaseibacillus paracasei
  source 1..1260: mol_type = other DNA
gtgttatccgttaaaatcaaccttttctttcaaaaagctttgtatcttatgcttctcttacttcaagtgaatttttttaacctatttggtagcccaaatttttatcaaatgaactcagataattcgaaagtgcttgttctttttttggttaccatttcggtttttatttgggtccctattgcgataactgccctttttaaagcaaaagagcggtcaaagcactcgtttaattggttgatcattggttttttgttttgttgggttgctgtcctctttggcagttcaagtgtgtatcaaattagcctaagaaaagcttttaatttcagttactactatccgattgtggcatacttctttccatttgcctggctcgttaaaagtgatttttcttttgtactcaagtcatttaaattttttgcatattttgagctcttgattttactgatacaagatctagttcttagtttaagtggaaagctttttcttagttttgatccttttggacaacaaatgtttatggattctggacgaatcatggcggggaccgactttcttttgttggcctgtttcattattgttttagccagaaaacttaaacacacgcttccgtcatatctagaagttttgttttttttagggttagtctttcacttgctctttttcacaaagagtagaatgctcctcctacttgtgatagctattttaagtgtagctattttctttaactcctccaaaggcttcacaatacctgttcgtttgatcttctatattttttgttttgttggtcttctagcgttgatgaatgtattgatcgccaagatgaattttttctccggcgacagagcggccagtggacaagttagacttcaggcgattgcttattatctaaacaatcttggaattaataaatggtttggttttggatttaccccatactctgatcaaattggtggaggcggccaaggcgtagatggcggcgttttttacaccagtgatgttggtatgatcggcttcattgcaatctttggagctctcggagtgctttttgctattttattcttatcaagttttgttcgatttttacgcacctttggtgacttttctgctaaattgattgtaattgtatacatttttggccagtggatttcactctcatcgtttgatatcagtagaattttgattttccctattgctctgggttttctgataggctttaaggaatttctcaattctagagagaacgtattagatgatagttaa

SEQ ID NO: 7 - DNA, 666 bp, Lacticaseibacillus paracasei
  source 1..666: mol_type = other DNA
atgccaacaacttctgattccctagcgattcttgacaaaattcaaatttatttttcggctttgtttaaagtgattcgtggctttttattgtctgtgacaacgcgccatgcaaagccactaatatttttgggacgacacgttaaaatcatgaatcggcagtatttacacatagaagcaaaagtaaagtttgaggattattgtgagattcaaggactatcaacaaatggactttattttgcgaaagacgtcactatcggccggggggttcaaattagaccttctagctattacggcgtaggccatattggctatggatttagtattggagagaatagttcagttgggccaggtggattcattggatgtgctggtaaggttcaaatcaataagaacgtaatgattggcccaaatgttacgattattgcagaaaatcatcattttcacagtacaaataaatcaataaaagatcaaggtgtttatcaaaaaggaatagtaatccatgatgatgtttggattggagcaaatgttactattttagacggtgtaacaatttgcagtggagcagttattggtgctggtgcaattattacaaaggatgtgccagctaatacaattttggttgataagttaaacccaattttgagaagccgaattgcccacagttag

SEQ ID NO: 8 - DNA, 1437 bp, Lacticaseibacillus paracasei
  source 1..1437: mol_type = genomic DNA
atgaaagttatcaaaaactttatttggaatgcaggatatcagatattcgtcctaatcgttcccttagtaacagtaccgtatattaatcgtattttaggtcccacgggggtcggaattaatgcttttactaattcaattgttcagtattttgttctttttggtagcttaggaattaatctgtatggtaatagaggaattgcatacagaagagacgataaagttgctttgacaaaatatttttgggaggtttctttccttcgttttatttcagtgggtgtagctgttattgcctatctgatattcacattttctatggacagatatcgaatattctatctggctcaaggctgtatgcttgtaggtgcggcatttgatatttcatggttctttcaaggactggaaaactttcgtgtcacggtggttcggaacgttttagtacggattgcctcacttgtcttaatttttttgttggtgcataaagcaagtgatacagcaatctatattttaatattgtccggttcgcagttacttggtaatttgacgttttggccatctttgcgtgctaacctgactcacttccctaaattgtcatctttgcaagtttggcaccacatgaagccagctttcctcttacttattccgcagctggcaatccagatttatgttcagttgaataaaactatgctaggaatcttgcagggtgtcacagcggcgggtttttatgagaattctgacaaaattataaaaatgttgttagcattggtgactgcaacaggcaccgttcttttaccacatgtcgcccattatttcgctagtggtaaccatgaagctgttaaacgttcattagcatcttcaatgcatgtgatattagtattggcatttcctcttgcttttggtatagctgctgtttcgacgccgttcacttatttctttttcagtgtcaagtttatgcctgtggccccgctgatggcagttgaggctatcgtcgtgataccgatttcgattgcaagtgctattggtgtacaatatttgttaccaactgatcaagttaaaccgtatacagtttcagttattttgggttcgttggttaatatcgttgttaatgtaccattgatcctttggttgggaacaatgggtgctgtgattggaacaattctttccgaatcggtggtaactctttatcaaatttacgctattaaaaaccaactttccctaggagaactattcagcgaatcgtggaagtattgtttgagcgcattgatcatgtttgctgtcataaaaggatggcaacacattttgacaataagcataacttcattgatattagaggttttgcttggtatgatcgtttacttcgttgttttattgttattacgtccgcgtattctgttcggctatatagggccttatatggggcgctttcgtaatcgaatatag

SEQ ID NO: 9 - DNA, 867 bp, Lacticaseibacillus paracasei
  source 1..867: mol_type = other DNA
atgttgaaaatagggttaattcttaattatcaaaattatcaacagacgattatctgttgtcttaatctaattaagagcggcgttgaccatgttttcattgttgacaatggttcgactaatgactctgtgcacgaacttcatgctgctcttgacaagtataagcaggtgcgcgtccttgctacaaaggccaatttagggtatgcacggggaaacaatgttggattgcgagcaattgaaagtgagtttgggttagctgacgatcacattctaatcgttgtcaatcctgatagtttgctcaattcagataacatcgaacaagttaccaacttctgtcttagtcatactgaagcgggcacagttactgtcccccaaaagggcaatcagaaaacagcatggcataacattactaagaaaagagcgcttttgtataattcacgtattttttcgaaatttgctcatcgttgtggaaaagaggaagcaattccataccaagtaagacactcggacactaaaagtatcaaagtggatgtcaatttaggtgctttttttgctattcgtcagacggttttctcgaaagtcggttactttgattcggccacttttctttactacgaagagcaagcactgacatttaagttacaagctcaaggatatcaaaattatttgcttttgacatcaagctatgttcacaaagggcagggatcaacacaattagcttcaagaaaggttctggggtattatcaacagagtagacgatatcttttgatacaatacttacacgcgggaaagtttgctcttcgtttttacgattggactattaggttcgaagatgtcttgagtggtgaccgtttttctgggaaggattga

SEQ ID NO: 10 - DNA, 717 bp, Lacticaseibacillus paracasei
  source 1..717: mol_type = other DNA
ttggggatcgtttctgccgcattttggcaatgtattggaggggtgaatttggagacaacatctagtcgtgaacaagttaatgccgagcaggttgaccttggggggttgacgccgagctacatattctcgaagcgttgctttgattttttggctagtctagttgggctgatcttacttagtggtgtatttctgatcattggaatcttaattaaagttgatgatccacatggaaagatattctattcgcagacccggcttggtaaaaatggccgagagtttcagatgtggaagtttcgatcgatggtgagtggcgctgacaagatggttgataagttgcttcgacgtaatgaggtccaaggtgccatgtttaagattaagaatgatcctcgtattacacgtgttggtcgtgttcttcggaagtatagtcttgacgagttacctcagctttataatgtcttggtcggggatatgagtttggttgggcctcgaccaccgctacctagagaagttgttaagtataccgattacgatcttcagcgacttgccgttattccgggctgtacaggtttgtggcaagtctcgggtcgaaatgagcttggcttttctgagatggttgcgttggacattcattatatcaacagtgcgtctttctttggagatctcaagattcttatgaaaacggtaatggttgtgattcatccgactggtgcctattga

SEQ ID NO: 11 - protein, 309 aa, Lacticaseibacillus paracasei
MNEQIDLSRLWNVFKRSFIAMVILGILCMVAAYFGAKTFIVPKYEADTSLLVNRKQDNDPNMQLNAQQADVQIINTYKDIITRPVVLQAVAGDLTSPRRVITKKAEKAVYGTRYNATTGIRERYVVEKAKPAQYKLKPAKYSNLTADDLAKMVSVSTQQNSQVFTVSVKDTDPIRARDIANEVAKVFKQKIAQIMSISNVSIVSEASANLSPVSPKLPLIALVGLLLGILVAFIWGLIRELTDQTIKDLDFITDDLGLVNLGIVNYVKRMKDMDQAIAKVKSENEESKDDESFEEFNMQDLPQRSRRRI

SEQ ID NO: 12 - protein, 252 aa, Lacticaseibacillus paracasei
MSLNGIFKKFTHRDEEDNETQKNGVMLVTFAEPKHVVAEQFRTVRTNIEFAGAALDRCEVVMFTSSSMSEGKSTVSANVAVTWAQAGEKVLLIDADLRRPTVHATFRTLNLEGVTTVLTGKTKPSDVVEKTFVDNLDIITSGPVPPNPSELLNSKRMANLLEWGRANYDIIVLDAPSVLAVSDVQVLVPKTDGVVVVTNMGKTLKGDLKRTVEVLKLAKAKILGSVERVRATKGDRGYGYGYGYGYQSNDER

SEQ ID NO: 13 - protein, 393 aa, Lacticaseibacillus paracasei
MTEKRKVFIIGSKGTPAKYGGFETFVDNLVSRQNSSQIKYFIACRRDLSDNKADLYDYKKATCFNVDVPNIGPAKAILYDLRALSWTLDYIQKNNIRGAIVYILACRVGPFLKHYSKRLKLYDTQIFVNPDGHEWMRAKWGFFVRKYWKLSERLMIKDADLIICDSKHIELYIREKYRSYKPKTIYSSYGADVATSQDVKAQDLQNWFNKKQISSGQYYLVVGRFVPENNYQTIVAEFEKSKTKKDLVIITNPDNTKFLKSLKDQTGFEKDNRIKFVGTVYDKDLLSAIRRNAFGYIHGHEVGGTNPSLLEALGTTNLNLLFDVGFNKEVGQDAAVYWNKQAGNLAHIINRVDQMSEEERQTLGKKAKQIIDKNFSWDKIVSQNERQFIDGKI

SEQ ID NO: 14 - protein, 385 aa, Lacticaseibacillus paracasei
MEKYKILFLHAGAELYGADKILLEIVENIDRKTFEPIVILPEDGPLVSKMREAGAEVSVLPYPILRRKFFNIRGIGNYIFSYIRFSRRLKKIVNKENIRLVHVNTTAVLEGVWLKLFTKAKIVWHVHEIIMKPKFIYKLICFLIQHFSDQAVAVSDATKQRLIDSGIVDKMKVITIHNGISKDYPQNGPDYVRKSLSISPDAVVIGMVGRVNAWKGQGDFIDAVGPILQKSQNVHALLVGSAYQGEEVYEHKLFDKVASLDTKERIHLCPFTEQIADYYSAFNIFVLPSIQPDPFPTVVLEAMSNSLPVVAYDHGGASEMIVDNETGYLCTALDVSELSRKLELLVGDRALRIKMGQKARVRQEAEFSLDQFVNRMTRVYLDLIE

SEQ ID NO: 15 - protein, 324 aa, Lacticaseibacillus paracasei
MTVNRKTDVSIIIPAHNAEPFITKCLQSIQQQSFHNFEVLVVENGSTDHTVESVLPFVSTDKRIRLLQNSDLGVSNARNLALQKAQSKFVTFVDADDYISNTHIQVLMDSVKDKEDDMGVTGFSYETEDGKILKVISVLNSKMSAEEAIRATYDLTGIQGIVSNKIFKKSIIDRYGIRFDPSISKYEDHKFVVAYLVHCQQVSCKSDITYHYIKHPESSLFTVKTSLIQDLDVFLSIRKMIVNHGFKDFKKYVNDPLQNIVLSHYWHPVDSHDKTEAAKRMVDRKFFSYNLLNMSIKNKLKCFFAFLSLGPYCIKRKFRNNDAS

SEQ ID NO: 16 - protein, 419 aa, Lacticaseibacillus paracasei
MLSVKINLFFQKALYLMLLLLQVNFFNLFGSPNFYQMNSDNSKVLVLFLVTISVFIWVPIAITALFKAKERSKHSFNWLIIGFLFCWVAVLFGSSSVYQISLRKAFNFSYYYPIVAYFFPFAWLVKSDFSFVLKSFKFFAYFELLILLIQDLVLSLSGKLFLSFDPFGQQMFMDSGRIMAGTDFLLLACFIIVLARKLKHTLPSYLEVLFFLGLVFHLLFFTKSRMLLLLVIAILSVAIFFNSSKGFTIPVRLIFYIFCFVGLLALMNVLIAKMNFFSGDRAASGQVRLQAIAYYLNNLGINKWFGFGFTPYSDQIGGGGQGVDGGVFYTSDVGMIGFIAIFGALGVLFAILFLSSFVRFLRTFGDFSAKLIVIVYIFGQWISLSSFDISRILIFPIALGFLIGFKEFLNSRENVLDDS

SEQ ID NO: 17 - protein, 221 aa, Lacticaseibacillus paracasei
MPTTSDSLAILDKIQIYFSALFKVIRGFLLSVTTRHAKPLIFLGRHVKIMNRQYLHIEAKVKFEDYCEIQGLSTNGLYFAKDVTIGRGVQIRPSSYYGVGHIGYGFSIGENSSVGPGGFIGCAGKVQINKNVMIGPNVTIIAENHHFHSTNKSIKDQGVYQKGIVIHDDVWIGANVTILDGVTICSGAVIGAGAIITKDVPANTILVDKLNPILRSRIAHS

SEQ ID NO: 18 - protein, 478 aa, Lacticaseibacillus paracasei
MKVIKNFIWNAGYQIFVLIVPLVTVPYINRILGPTGVGINAFTNSIVQYFVLFGSLGINLYGNRGIAYRRDDKVALTKYFWEVSFLRFISVGVAVIAYLIFTFSMDRYRIFYLAQGCMLVGAAFDISWFFQGLENFRVTVVRNVLVRIASLVLIFLLVHKASDTAIYILILSGSQLLGNLTFWPSLRANLTHFPKLSSLQVWHHMKPAFLLLIPQLAIQIYVQLNKTMLGILQGVTAAGFYENSDKIIKMLLALVTATGTVLLPHVAHYFASGNHEAVKRSLASSMHVILVLAFPLAFGIAAVSTPFTYFFFSVKFMPVAPLMAVEAIVVIPISIASAIGVQYLLPTDQVKPYTVSVILGSLVNIVVNVPLILWLGTMGAVIGTILSESVVTLYQIYAIKNQLSLGELFSESWKYCLSALIMFAVIKGWQHILTISITSLILEVLLGMIVYFVVLLLLRPRILFGYIGPYMGRFRNRI

SEQ ID NO: 19 - protein, 288 aa, Lacticaseibacillus paracasei
MLKIGLILNYQNYQQTIICCLNLIKSGVDHVFIVDNGSTNDSVHELHAALDKYKQVRVLATKANLGYARGNNVGLRAIESEFGLADDHILIVVNPDSLLNSDNIEQVTNFCLSHTEAGTVTVPQKGNQKTAWHNITKKRALLYNSRIFSKFAHRCGKEEAIPYQVRHSDTKSIKVDVNLGAFFAIRQTVFSKVGYFDSATFLYYEEQALTFKLQAQGYQNYLLLTSSYVHKGQGSTQLASRKVLGYYQQSRRYLLIQYLHAGKFALRFYDWTIRFEDVLSGDRFSGKD

SEQ ID NO: 20 - protein, 238 aa, Lacticaseibacillus paracasei
MGIVSAAFWQCIGGVNLETTSSREQVNAEQVDLGGLTPSYIFSKRCFDFLASLVGLILLSGVFLIIGILIKVDDPHGKIFYSQTRLGKNGREFQMWKFRSMVSGADKMVDKLLRRNEVQGAMFKIKNDPRITRVGRVLRKYSLDELPQLYNVLVGDMSLVGPRPPLPREVVKYTDYDLQRLAVIPGCTGLWQVSGRNELGFSEMVALDIHYINSASFFGDLKILMKTVMVVIHPTGAY

SEQ ID NO: 21 - DNA, 37 bp, Lacticaseibacillus paracasei
  source 1..37: mol_type = other DNA
cactgcgaaaaaaatctaactctttccccacctaatc

SEQ ID NO: 22 - DNA, 39 bp, Lacticaseibacillus paracasei
  source 1..39: mol_type = other DNA
ctgcaggtcgactctagagcaatcaacgtgtagtaatgc

SEQ ID NO: 23 - DNA, 42 bp, Lacticaseibacillus paracaseic
  source 1..42: mol_type = other DNA
acccggggatcctctagagaccataatcattctttttgagtg

SEQ ID NO: 24 - DNA, 46 bp, Lacticaseibacillus paracasei
  source 1..46: mol_type = other DNA
gggattaggtggggaaagagttagatttttttcgcagtgtaaaaag

SEQ ID NO: 25 - DNA, 23 bp, Lacticaseibacillus paracasei
  source 1..23: mol_type = other DNA
tttgatatagactccgttatcgg

SEQ ID NO: 26 - DNA, 21 bp, Lacticaseibacillus paracasei
  source 1..21: mol_type = other DNA
tcattctgacgggtttatagg

SEQ ID NO: 27 - DNA, 20 bp, Lacticaseibacillus paracasei
  source 1..20: mol_type = other DNA
ttaagttgggtaacgccagg

SEQ ID NO: 28 - DNA, 21 bp, Lacticaseibacillus paracasei
  source 1..21: mol_type = other DNA
ggataacaatttcacacagga

SEQ ID NO: 29 - DNA, 20 bp, Lacticaseibacillus paracasei
  source 1..20: mol_type = other DNA
cgattgtcaccaaaaacatc

SEQ ID NO: 30 - DNA, 21 bp, Lacticaseibacillus paracasei
  source 1..21: mol_type = other DNA
ggaagggatacaccctaaatc

SEQ ID NO: 31 - DNA, 28 bp, Lacticaseibacillus paracasei
  source 1..28: mol_type = other DNA
taacccgggtggacttgattacacaagc

SEQ ID NO: 32 - DNA, 28 bp, Lacticaseibacillus paracasei
  source 1..28: mol_type = other DNA
taactgcagacactctttttacactgcg